European Patent Specification EP 3 837 366 B1, published February 18, 2026. Title: HEPATITS B VIRUS (HBV) dsRNA AGENT COMPOSITIONS AND METHODS OF USE THEREOF. Applicant: Alnylam Pharmaceuticals, Inc. Jadhav, Vasant R. Maier, Martin A. Milstein, Stuart Schlegel, Mark K. Application PCT. The sequence listing filed with the application follows.

SEQUENCE LISTING (49 sequences)

SEQ ID NO: 1 - DNA, 3215 bp, Hepatitis B virus
  NC_003977.1, Hepatitis B virus, complete genome
ctccacaacattccaccaagctctgctagatcccagagtgaggggcctatattttcctgctggtggctccagttccggaacagtaaaccctgttccgactactgcctcacccatatcgtcaatcttctcgaggactggggaccctgcaccgaacatggagagcacaacatcaggattcctaggacccctgctcgtgttacaggcggggtttttcttgttgacaagaatcctcacaataccacagagtctagactcgtggtggacttctctcaattttctagggggagcacccacgtgtcctggccaaaattcgcagtccccaacctccaatcactcaccaacctcttgtcctccaacttgtcctggctatcgctggatgtgtctgcggcgttttatcatattcctcttcatcctgctgctatgcctcatcttcttgttggttcttctggactaccaaggtatgttgcccgtttgtcctctacttccaggaacatcaactaccagcacgggaccatgcagaacctgcacgattcctgctcaaggaacctctatgtttccctcttgttgctgtacaaaaccttcggacggaaactgcacttgtattcccatcccatcatcctgggctttcgcaagattcctatgggagtgggcctcagtccgtttctcctggctcagtttactagtgccatttgttcagtggttcgtagggctttcccccactgtttggctttcagctatatggatgatgtggtattgggggccaagtctgtacaacatcttgagtccctttttacctctattaccaattttcttttgtctttgggtatacatttgaaccctaataaaaccaaacgttggggctactcccttaacttcatgggatatgtaattggaagttggggtactttaccgcaggaacatattgtacaaaaactcaagcaatgttttcgaaaattgcctgtaaatagacctattgattggaaagtatgtcaaagaattgtgggtcttttgggctttgctgccccttttacacaatgtggctatcctgccttgatgcctttatatgcatgtatacaatctaagcaggctttcactttctcgccaacttacaaggcctttctgtgtaaacaatatctaaacctttaccccgttgcccggcaacggtcaggtctctgccaagtgtttgctgacgcaacccccacgggttggggcttggccataggccatcggcgcatgcgtggaacctttgtggctcctctgccgatccatactgcggaactcctagcagcttgttttgctcgcagccggtctggagcgaaacttatcggaaccgacaactcagttgtcctctctcggaaatacacctcctttccatggctgctaggctgtgctgccaactggatcctgcgcgggacgtcctttgtctacgtcccgtcggcgctgaatcccgcggacgacccgtctcggggccgtttgggcctctaccgtccccttcttcatctgccgttccggccgaccacggggcgcacctctctttacgcggtctccccgtctgtgccttctcatctgccggaccgtgtgcacttcgcttcacctctgcacgtagcatggagaccaccgtgaacgcccaccaggtcttgcccaaggtcttacacaagaggactcttggactctcagcaatgtcaacgaccgaccttgaggcatacttcaaagactgtttgtttaaagactgggaggagttgggggaggagattaggttaaaggtctttgtactaggaggctgtaggcataaattggtctgttcaccagcaccatgcaactttttcccctctgcctaatcatctcatgttcatgtcctactgttcaagcctccaagctgtgccttgggtggctttggggcatggacattgacccgtataaagaatttggagcttctgtggagttactctcttttttgccttctgacttctttccttctattcgagatctcctcgacaccgcctctgctctgtatcgggaggccttagagtctccggaacattgttcacctcaccatacagcactcaggcaagctattctgtgttggggtgagttgatgaatctggccacctgggtgggaagtaatttggaagacccagcatccagggaattagtagtcagctatgtcaatgttaatatgggcctaaaaattagacaactattgtggtttcacatttcctgccttacttttggaagagaaactgtccttgagtatttggtgtcttttggagtgtggattcgcactcctcccgcttacagaccaccaaatgcccctatcttatcaacacttccggaaactactgttgttagacgacgaggcaggtcccctagaagaagaactccctcgcctcgcagacgaaggtctcaatcgccgcgtcgcagaagatctcaatctcgggaatctcaatgttagtatcccttggactcataaggtgggaaactttactgggctttattcttctactgtacctgtctttaatcctgattggaaaactccctcctttcctcacattcatttacaggaggacattattaatagatgtcaacaatatgtgggccctctgacagttaatgaaaaaaggagattaaaattaattatgcctgctaggttctatcctaaccttaccaaatatttgcccttggacaaaggcattaaaccgtattatcctgaatatgcagttaatcattacttcaaaactaggcattatttacatactctgtggaaggctggcattctatataagagagaaactacacgcagcgcctcattttgtgggtcaccatattcttgggaacaagagctacagcatgggaggttggtcttccaaacctcgacaaggcatggggacgaatctttctgttcccaatcctctgggattctttcccgatcaccagttggaccctgcgttcggagccaactcaaacaatccagattgggacttcaaccccaacaaggatcactggccagaggcaaatcaggtaggagcgggagcatttggtccagggttcaccccaccacacggaggccttttggggtggagccctcaggctcagggcatattgacaacactgccagcagcacctcctcctgcctccaccaatcggcagtcaggaagacagcctactcccatctctccacctctaagagacagtcatcctcaggccatgcagtggaa

SEQ ID NO: 2 - DNA, 3215 bp, Artificial Sequence
  Reverse Complement of SEQ ID NO:1
ttccactgcatggcctgaggatgactgtctcttagaggtggagagatgggagtaggctgtcttcctgactgccgattggtggaggcaggaggaggtgctgctggcagtgttgtcaatatgccctgagcctgagggctccaccccaaaaggcctccgtgtggtggggtgaaccctggaccaaatgctcccgctcctacctgatttgcctctggccagtgatccttgttggggttgaagtcccaatctggattgtttgagttggctccgaacgcagggtccaactggtgatcgggaaagaatcccagaggattgggaacagaaagattcgtccccatgccttgtcgaggtttggaagaccaacctcccatgctgtagctcttgttcccaagaatatggtgacccacaaaatgaggcgctgcgtgtagtttctctcttatatagaatgccagccttccacagagtatgtaaataatgcctagttttgaagtaatgattaactgcatattcaggataatacggtttaatgcctttgtccaagggcaaatatttggtaaggttaggatagaacctagcaggcataattaattttaatctccttttttcattaactgtcagagggcccacatattgttgacatctattaataatgtcctcctgtaaatgaatgtgaggaaaggagggagttttccaatcaggattaaagacaggtacagtagaagaataaagcccagtaaagtttcccaccttatgagtccaagggatactaacattgagattcccgagattgagatcttctgcgacgcggcgattgagaccttcgtctgcgaggcgagggagttcttcttctaggggacctgcctcgtcgtctaacaacagtagtttccggaagtgttgataagataggggcatttggtggtctgtaagcgggaggagtgcgaatccacactccaaaagacaccaaatactcaaggacagtttctcttccaaaagtaaggcaggaaatgtgaaaccacaatagttgtctaatttttaggcccatattaacattgacatagctgactactaattccctggatgctgggtcttccaaattacttcccacccaggtggccagattcatcaactcaccccaacacagaatagcttgcctgagtgctgtatggtgaggtgaacaatgttccggagactctaaggcctcccgatacagagcagaggcggtgtcgaggagatctcgaatagaaggaaagaagtcagaaggcaaaaaagagagtaactccacagaagctccaaattctttatacgggtcaatgtccatgccccaaagccacccaaggcacagcttggaggcttgaacagtaggacatgaacatgagatgattaggcagaggggaaaaagttgcatggtgctggtgaacagaccaatttatgcctacagcctcctagtacaaagacctttaacctaatctcctcccccaactcctcccagtctttaaacaaacagtctttgaagtatgcctcaaggtcggtcgttgacattgctgagagtccaagagtcctcttgtgtaagaccttgggcaagacctggtgggcgttcacggtggtctccatgctacgtgcagaggtgaagcgaagtgcacacggtccggcagatgagaaggcacagacggggagaccgcgtaaagagaggtgcgccccgtggtcggccggaacggcagatgaagaaggggacggtagaggcccaaacggccccgagacgggtcgtccgcgggattcagcgccgacgggacgtagacaaaggacgtcccgcgcaggatccagttggcagcacagcctagcagccatggaaaggaggtgtatttccgagagaggacaactgagttgtcggttccgataagtttcgctccagaccggctgcgagcaaaacaagctgctaggagttccgcagtatggatcggcagaggagccacaaaggttccacgcatgcgccgatggcctatggccaagccccaacccgtgggggttgcgtcagcaaacacttggcagagacctgaccgttgccgggcaacggggtaaaggtttagatattgtttacacagaaaggccttgtaagttggcgagaaagtgaaagcctgcttagattgtatacatgcatataaaggcatcaaggcaggatagccacattgtgtaaaaggggcagcaaagcccaaaagacccacaattctttgacatactttccaatcaataggtctatttacaggcaattttcgaaaacattgcttgagtttttgtacaatatgttcctgcggtaaagtaccccaacttccaattacatatcccatgaagttaagggagtagccccaacgtttggttttattagggttcaaatgtatacccaaagacaaaagaaaattggtaatagaggtaaaaagggactcaagatgttgtacagacttggcccccaataccacatcatccatatagctgaaagccaaacagtgggggaaagccctacgaaccactgaacaaatggcactagtaaactgagccaggagaaacggactgaggcccactcccataggaatcttgcgaaagcccaggatgatgggatgggaatacaagtgcagtttccgtccgaaggttttgtacagcaacaagagggaaacatagaggttccttgagcaggaatcgtgcaggttctgcatggtcccgtgctggtagttgatgttcctggaagtagaggacaaacgggcaacataccttggtagtccagaagaaccaacaagaagatgaggcatagcagcaggatgaagaggaatatgataaaacgccgcagacacatccagcgatagccaggacaagttggaggacaagaggttggtgagtgattggaggttggggactgcgaattttggccaggacacgtgggtgctccccctagaaaattgagagaagtccaccacgagtctagactctgtggtattgtgaggattcttgtcaacaagaaaaaccccgcctgtaacacgagcaggggtcctaggaatcctgatgttgtgctctccatgttcggtgcagggtccccagtcctcgagaagattgacgatatgggtgaggcagtagtcggaacagggtttactgttccggaactggagccaccagcaggaaaatataggcccctcactctgggatctagcagagcttggtggaatgttgtggag

SEQ ID NO: 3 - DNA, 3215 bp, Hepatitis B virus
  AB014381.1, Hepatitis B virus genomic DNA, complete sequence, isolate 22Y04HCC
  misc_feature (1)...(3215): n = A,T,C or G
ctccaccacattccaccaagctctgctacaccccagagtaaggggcctatactttcctgctggtggctccagttccggaacagtaaaccctgttccgactactgcctctcccatatcgtcaatcttctcgaggactggggaccctgcaccgaacatggagaacacaacatcaggattcctaggacccctgctcgtgttacaggcggggtttttcttgttgacaagaatcctcacaataccacagagtctagactcgtggtggacttctctcaattttctagggggagcacccacgtgtcctggccaaaattcgcagtccccaacctccaatcactcaccaacctcttgtcctccaatttgtcctggctatcgctggatgtgtctgcggcgttttatcatattcctcttcatcctgctgctatgcctcatcttcttgttggttcttctggactaccaaggtatgttgcccgtttgtcctctacttccaggaacatcaactaccagcacgggaccatgcaagacctgcacgattcctgctcaaggcacctctatgtttccctcttgttgctgtacaaaaccttcggacggaaactgcacttgtattcccatcccatcatcctgggctttcgcaagattcctatgggagtgggcctcagtccgtttctcctggctcagtttactagtgccatttgttcagtggttcgtagggctttcccccactgtttggctttcagttatatggatgatgtggtattgggggccaagtctgtacaacatcttgagtccctttttaccgctgttaccaattttcttttgtctttgggtatacatttgaaccctaataaaaccaaacgttggggttactcccttaacttcatgggatatgtaattggaagttggggtactttaccgcaagaccatattgtactaaaaatcaagcaatgttttcgaaaactgcctgtaaatagacctattgattggaaagtatgtcagagaattgtgggtcttttgggctttgctgccccttttacacaatgtggctatcctgccttaatgcctttatatgcatgtatacaatctaagcaggctttcactttctcgccaacttacaaggcctttctgtgtaaacaatatctgaacctttaccccgttgcccggcaacggtcaggtctctgccaagtgtttgctgacgcaacccccactggatggggcttggctattggccatcgccgcatgcgtggaacctttgtggctcctctgccgatccatactgcggaactcctagcagcttgttttgctcgcagccggtctggagcgaaactgatcggaacggacaactctgttgttctctctcggaaatacacctcctttccatggctgctagggtgtgctgccaactggatcctgcgcgggacgtcctttgtttacgtcccgtcggcgctgaatcccgcggacgacccatctcggggccgtttgggtctctaccgtccccttcttcatctgccgttccggccgaccacggggcgcacctctctttacgcggtctccccgtctgtgccttctcatctgccggaccgtgtgcacttcgcttcacctctgcacgtcgcatggagaccaccgtgaacgcccaccaggtcttgcccaaggtcttatataagaggactcttggactctcagcaatgtcaacgaccgaccttgaggcatacttcaaagactgtttgtttaaggactgggaggagttgggggaggagattaggttaatgatctttgtactaggaggctgtaggcataaattggtctgttcaccagcaccatgcaactttttcacctctgcctaatcatctcatgttcatgtcctactgttcaagcctccaagctgtgccttgggtggctttaggacatggacattgacccatataaagaatttggagcttctgtggagttactctcttttttgccttctgacttttttccttctattcgagatctcctcgacaccgcctctgctctgtatcgggaggccttagagtctccggaacattgttcacctcaccatacagcactcagacaagccattctgtgttggggtgagttgatgaatctggccacctgggtgggaagtaatttggaagacccagcatccagggaattagtagtcagctatgtcaatgttaatatgggcctaaaaatcagacaactactgtggtttcacatttcctgtcttacttttggaagagaaactgttcttgagtatttggtgtcttttggagtgtggattcgcactcctcctgcttacagaccatcaaatgcccctatcttatcaacacttccggaaactactgttgttagacgacgaggcaggtcccctagaagaagaactccctcgcctcgcagacgaaggtctcaatcgccgcgtcgcagaagatctcaatctcgggaacctcaatgttagtatcccttggactcataaggtgggaaactttactgggctttattcttctactgtacctgtctttaatcctgagtggcaaactccctcttttcctcatattcatttgcaggaggacattattaatagatgtcaacaatatgtgggccctcttacagttaatgaaaaaaggagattaaaattaattatgcctgctaggttctatcctaaccttaccaaatatttgcccttggacaaaggcattaaaccatattatccggaacatgcagttaatcattacttcaaaactaggcattatttacatactctgtggaaggcnggcattctatataagagagaaactacacgcagcgcctcattttgtgggtcaccatattcttgggaacaagagctacagcatgggaggttggtcttccaaacctcgacaaggcatggggacaaatctttctgttcccaatcctctgggattctttcccgatcaccagttggaccctgcgttcggagccaactcaaacaatccagattgggacttcaaccccaacaaggatcactggccagaggcaaatcaggtaggagcgggagcattcgggccagggttcaccccaccacacggcggtcttttggggtggagccctcaggctcagggcacattgacaacagtgccagtagcacctcctcctgcctccaccaatcggcagtcaggaagacagcctactcccatctctccacctctaagagacagtcatcctcaggccatgcagtggaa

SEQ ID NO: 4 - DNA, 3215 bp, Artificial Sequence
  Reverse Complement of SEQ ID NO:3
  misc_feature (1)...(3215): n = A,T,C or G
ttccactgcatggcctgaggatgactgtctcttagaggtggagagatgggagtaggctgtcttcctgactgccgattggtggaggcaggaggaggtgctactggcactgttgtcaatgtgccctgagcctgagggctccaccccaaaagaccgccgtgtggtggggtgaaccctggcccgaatgctcccgctcctacctgatttgcctctggccagtgatccttgttggggttgaagtcccaatctggattgtttgagttggctccgaacgcagggtccaactggtgatcgggaaagaatcccagaggattgggaacagaaagatttgtccccatgccttgtcgaggtttggaagaccaacctcccatgctgtagctcttgttcccaagaatatggtgacccacaaaatgaggcgctgcgtgtagtttctctcttatatagaatgccngccttccacagagtatgtaaataatgcctagttttgaagtaatgattaactgcatgttccggataatatggtttaatgcctttgtccaagggcaaatatttggtaaggttaggatagaacctagcaggcataattaattttaatctccttttttcattaactgtaagagggcccacatattgttgacatctattaataatgtcctcctgcaaatgaatatgaggaaaagagggagtttgccactcaggattaaagacaggtacagtagaagaataaagcccagtaaagtttcccaccttatgagtccaagggatactaacattgaggttcccgagattgagatcttctgcgacgcggcgattgagaccttcgtctgcgaggcgagggagttcttcttctaggggacctgcctcgtcgtctaacaacagtagtttccggaagtgttgataagataggggcatttgatggtctgtaagcaggaggagtgcgaatccacactccaaaagacaccaaatactcaagaacagtttctcttccaaaagtaagacaggaaatgtgaaaccacagtagttgtctgatttttaggcccatattaacattgacatagctgactactaattccctggatgctgggtcttccaaattacttcccacccaggtggccagattcatcaactcaccccaacacagaatggcttgtctgagtgctgtatggtgaggtgaacaatgttccggagactctaaggcctcccgatacagagcagaggcggtgtcgaggagatctcgaatagaaggaaaaaagtcagaaggcaaaaaagagagtaactccacagaagctccaaattctttatatgggtcaatgtccatgtcctaaagccacccaaggcacagcttggaggcttgaacagtaggacatgaacatgagatgattaggcagaggtgaaaaagttgcatggtgctggtgaacagaccaatttatgcctacagcctcctagtacaaagatcattaacctaatctcctcccccaactcctcccagtccttaaacaaacagtctttgaagtatgcctcaaggtcggtcgttgacattgctgagagtccaagagtcctcttatataagaccttgggcaagacctggtgggcgttcacggtggtctccatgcgacgtgcagaggtgaagcgaagtgcacacggtccggcagatgagaaggcacagacggggagaccgcgtaaagagaggtgcgccccgtggtcggccggaacggcagatgaagaaggggacggtagagacccaaacggccccgagatgggtcgtccgcgggattcagcgccgacgggacgtaaacaaaggacgtcccgcgcaggatccagttggcagcacaccctagcagccatggaaaggaggtgtatttccgagagagaacaacagagttgtccgttccgatcagtttcgctccagaccggctgcgagcaaaacaagctgctaggagttccgcagtatggatcggcagaggagccacaaaggttccacgcatgcggcgatggccaatagccaagccccatccagtgggggttgcgtcagcaaacacttggcagagacctgaccgttgccgggcaacggggtaaaggttcagatattgtttacacagaaaggccttgtaagttggcgagaaagtgaaagcctgcttagattgtatacatgcatataaaggcattaaggcaggatagccacattgtgtaaaaggggcagcaaagcccaaaagacccacaattctctgacatactttccaatcaataggtctatttacaggcagttttcgaaaacattgcttgatttttagtacaatatggtcttgcggtaaagtaccccaacttccaattacatatcccatgaagttaagggagtaaccccaacgtttggttttattagggttcaaatgtatacccaaagacaaaagaaaattggtaacagcggtaaaaagggactcaagatgttgtacagacttggcccccaataccacatcatccatataactgaaagccaaacagtgggggaaagccctacgaaccactgaacaaatggcactagtaaactgagccaggagaaacggactgaggcccactcccataggaatcttgcgaaagcccaggatgatgggatgggaatacaagtgcagtttccgtccgaaggttttgtacagcaacaagagggaaacatagaggtgccttgagcaggaatcgtgcaggtcttgcatggtcccgtgctggtagttgatgttcctggaagtagaggacaaacgggcaacataccttggtagtccagaagaaccaacaagaagatgaggcatagcagcaggatgaagaggaatatgataaaacgccgcagacacatccagcgatagccaggacaaattggaggacaagaggttggtgagtgattggaggttggggactgcgaattttggccaggacacgtgggtgctccccctagaaaattgagagaagtccaccacgagtctagactctgtggtattgtgaggattcttgtcaacaagaaaaaccccgcctgtaacacgagcaggggtcctaggaatcctgatgttgtgttctccatgttcggtgcagggtccccagtcctcgagaagattgacgatatgggagaggcagtagtcggaacagggtttactgttccggaactggagccaccagcaggaaagtataggccccttactctggggtgtagcagagcttggtggaatgtggtggag

SEQ ID NO: 5 - DNA, 1200 bp, Artificial Sequence
  psiCHECK2-HBV plasmid
ctccacaacattccaccaagctctgcaagatcccagagtcaggggcctgtattttcctgctggtggctccagttcaggaacagtgaaccctgttccgactattgcctctcccatatcgtcaatcttctcgaggactggggaccctgcaccgaacatggagaacatcacatcaggattcctaggacccctgctcgtgttacaggcggggtttttcttgttgacaaaaatcctcacaataccacagagtctagactcgtggtggacttctctcaattttctagggggagcacccgtgtgtcctggccaaaattcgcagtccccaacctccaatcactcaccaacctcctgtcctccaacttgtcctggctatcgttggatgtgtctgcggcgttttatcatcttcctcttcatcctgctgctatgcctcatcttcttgttggttcttctggactatcaaggtatgttgcccgtttgtcctctaattccaggatcatcaaccaccagcacgggaccatgcaaaacctgcacgactcctgctcaaggaacctctatgtttccctcatgttgctgtacaaaaccttcggacggaaattgcacctgtattcccatcccatcatcttgggctttcgcaaaatacctatgggagtgggcctcagtccgtttctcttggctcagtttactagtgccatttgttcagtggttcgtagggctttcccccactgtctggctttcagttatatggatgatgtggtattgggggccaagtctgtacagcatcttgagtccctttataccgctgttaccaattttcttttgtctttgggtatacatttaaaccctaacaaaacaaaaagatggggttattccctaaacttcatgggttatgtaattggaagttgggggacattgccacaggaacatattgtacaaaaaatcaaacaatgttttagaaaacttcctgttaacaggcctattgattggaaagtatgtcaacgaattgtgggtcttttgggctttgctgccccttttacacaatgtggttatcctgctttaatgcctttgtatgcatgtatacaagctaaacaggcttttactttctcgccaacttacaaggcctttctctgtaaacaatacatgaacctttaccccgttgctcggcaacggccaggtctgtgccaagtgtttgctgacgcaaccccc

SEQ ID NO: 6 - DNA, 681 bp, Hepatitis B virus
  HBV, genotype A
atggagaacatcacatcaggattcctaggacccctgctcgtgttacaggcggggtttttcttgttgacaagaatcctcacaataccgcagagtctagactcgtggtggacttctctcaattttctagggggatcacccgtgtgtcttggccaaaattcgcagtccccaacctccaatcactcaccaacctcctgtcctccaatttgtcctggttatcgctggatgtgtctgcggcgttttatcatattcctcttcatcctgctgctatgcctcatcttcttattggttcttctggattatcaaggtatgttgcccgtttgtcctctaattccaggatcaacaacaaccagtacgggaccatgcaaaacctgcacgactcctgctcaaggcaactctatgtttccctcatgttgctgtacaaaacctacggatggaaattgcacctgtattcccatcccatcgtcctgggctttcgcaaaatacctatgggagtgggcctcagtccgtttctcttggctcagtttactagtgccatttgttcagtggttcgtagggctttcccccactgtttggctttcagctatatggatgatgtggtattgggggccaagtctgtacagcatcgtgagtccctttataccgctgttaccaattttcttttgtctctgggtatacatttaa

SEQ ID NO: 7 - DNA, 681 bp, Hepatitis B virus
  HBV, genotype C
atggagaacacaacatcaggattcctaggacccctgctcgtgttacaggcggggtttttcttgttgacaagaatcctcacaataccacagagtctagactcgtggtggacttctctcaattttctagggggagcacccacgtgtcctggccaaaattcgcagtccccaacctccaatcactcaccaacctcttgtcctccaatttgtcctggctatcgctggatgtgtctgcggcgttttatcatattcctcttcatcctgctgctatgcctcatcttcttgttggttcttctggactaccaaggtatgttgcccgtttgtcctctacttccaggaacatcaactaccagcacgggaccatgcaagacctgcacgattcctgctcaaggaacctctatgtttccctcttgttgctgtacaaaaccttcggacggaaactgcacttgtattcccatcccatcatcctgggctttcgcaagattcctatgggagtgggcctcagtccgtttctcctggctcagtttactagtgccatttgttcagtggttcgtagggctttcccccactgtttggctttcagttatatggatgatgtggtattgggggccaagtctgtacaacatcttgagtccctttttacctctattaccaattttcttttgtctttgggtatacatttga

SEQ ID NO: 8 - DNA, 681 bp, Hepatitis B virus
  HBV, genotype E
atggaaagcatcacatcaggattcctaggacccctgctcgtgttacaggcggggtttttcttgttgacaaaaatcctcacaataccgcagagtctagactcgtggtggacttctctcaattttctagggggagctcccgtgtgtcttggccaaaattcgcagtccccaacctccaatcactcaccaacctcttgtcctccaatttgtcctggctatcgctggatgtgtctgcggcgttttatcatcttcctcttcatcctgctgctatgcctcatcttcttgttggttcttctggactatcaaggtatgttgcccgtttgtcctctaattccaggatcatcaaccaccagtacgggaccctgccgaacctgcacgactcttgctcaaggaacctctatgtttccctcatgttgctgttcaaaaccttcggacggaaattgcacttgtattcccatcccatcatcatgggctttcggaaaattcctatgggagtgggcctcagcccgtttctcctggctcagtttactagtgccatttgttcagtggttcgccgggctttcccccactgtctggctttcagttatatggatgatgtggtattgggggccaagtctgtacaacatcttgagtccctttatacctctgttaccaattttcttttgtctttgggtatacatttaa

SEQ ID NO: 9 - DNA, 681 bp, Hepatitis B virus
  HBV, genotype F
atggacaacatcacatcaggactcctaggacccctgctcgtgttacaggcggtgtgtttcttgttgacaaaaatcctcacaataccacagagtctagactcgtggtggacttctctcaattttctagggggactacccgggtgtcctggccaaaattcgcagtccccaacctccaatcacttaccaacctcctgtcctccaacttgtcctggctatcgttggatgtgtctgcggcgttttatcatcttcctcttcatcctgctgctatgcctcatcttcttgttggttcttctggactatcaaggtatgttgcccgtttgtcctctacttccaggatccacgaccaccagcacgggaccatgcaaaacctgcacaactcttgctcaaggaacctctatgtttccctcctgttgctgttccaaaccctcggacggaaactgcacctgtattcccatcccatcatcttgggctttaggaaaatacctatgggagtgggcctcagcccgtttctcctggctcagtttactagtgcaatttgttcagtggtgcgtagggctttcccccactgtctggcttttagttatatggatgatctggtattgggggccaaatctgtgcagcatcttgagtccctttataccgctgttaccaattttctgttatctgtgggtatccatttaa

SEQ ID NO: 10 - RNA, 19 nt, Artificial Sequence
  Synthetic oligonucleotide (sense)
gugugcacuucgcuucaca

SEQ ID NO: 11 - DNA, 19 bp, Artificial Sequence
  Synthetic oligonucleotide (sense)
gugugcactucgcuucaca

SEQ ID NO: 12 - DNA, 19 bp, Artificial Sequence
  Synthetic oligonucleotide (sense)
gugugcactucgcuucaca

SEQ ID NO: 13 - RNA, 21 nt, Artificial Sequence
  AD-66810 Antisense
ugugaagcgaagugcacacuu

SEQ ID NO: 14 - RNA, 21 nt, Artificial Sequence
  AD-192282 Antisense
ugugaagcgaagugcacacuu

SEQ ID NO: 15 - RNA, 21 nt, Artificial Sequence
  AD-192289 Antisense
ugugaagcgaagugcacacuu

SEQ ID NO: 16 - RNA, 21 nt, Artificial Sequence
  AD-81890 Antisense
ugugaagcgaagugcacacuu

SEQ ID NO: 17 - RNA, 21 nt, Artificial Sequence
  AD-81892 Antisense
ugugaagcgaagugcacacuu

SEQ ID NO: 18 - RNA, 21 nt, Artificial Sequence
  AD-192283 Antisense
ugugaagcgaagugcacacuu

SEQ ID NO: 19 - RNA, 21 nt, Artificial Sequence
  AD-192291 Antisense
ugugaagcgaagugcacacuu

SEQ ID NO: 20 - RNA, 21 nt, Artificial Sequence
  AD-192277 Antisense
ugugaagcgaagugcacacuu

SEQ ID NO: 21 - RNA, 21 nt, Artificial Sequence
  AD-192284 Antisense
ugugaagcgaagugcacacuu

SEQ ID NO: 22 - RNA, 21 nt, Artificial Sequence
  AD-192285 Antisense
ugugaagcgaagugcacacuu

SEQ ID NO: 23 - RNA, 21 nt, Artificial Sequence
  AD-192293 Antisense
ugugaagcgaagugcacacuu

SEQ ID NO: 24 - RNA, 21 nt, Artificial Sequence
  AD-192279 Antisense
ugugaagcgaagugcacacuu

SEQ ID NO: 25 - RNA, 21 nt, Artificial Sequence
  AD-192294 Antisense
ugugaagcgaagugcacacuu

SEQ ID NO: 26 - RNA, 21 nt, Artificial Sequence
  AD-192280 Antisense
ugugaagcgaagugcacacuu

SEQ ID NO: 27 - RNA, 21 nt, Artificial Sequence
  AD-192287 Antisense
ugugaagcgaagugcacacuu

SEQ ID NO: 28 - RNA, 21 nt, Artificial Sequence
  AD-192281 Antisense
ugugaagcgaagugcacacuu

SEQ ID NO: 29 - RNA, 19 nt, Artificial Sequence
  Synthetic oligonucleotide (sense)
gugugcacuucgcuucaca

SEQ ID NO: 30 - DNA, 19 bp, Artificial Sequence
  Synthetic oligonucleotide (sense)
gugugcactucgcuucaca

SEQ ID NO: 31 - DNA, 19 bp, Artificial Sequence
  Synthetic oligonucleotide (sense)
gugugcactucgcuucaca

SEQ ID NO: 32 - protein, 832 aa, Hepatitis B virus
  HBV P protein (YP_009173866)
MPLSYQHFRRLLLLDDEAGPLEEELPRLADEGLNRRVAEDLNLGNLNVSIPWTHKVGNFTGLYSSTVPVFNPHWKTPSFPNIHLHQDIIKKCEQFVGPLTVNEKRRLQLIMPARFYPKVTKYLPLDKGIKPYYPEHLVNHYFQTRHYLHTLWKAGILYKRETTHSASFCGSPYSWEQDLQHGAESFHQQSSGILSRPPVGSSLQSKHRKSRLGLQSQQGHLARRQQGRSWSIRAGFHPTARRPFGVEPSGSGHTTNFASKSASCLHQSPVRKAAYPAVSTFEKHSSSGHAVEFHNLPPNSARSQSERPVFPCWWLQFRNSKPCSDYCLSLIVNLLEDWGPCAEHGEHHIRIPRTPSRVTGGVFLVDKNPHNTAESRLVVDFSQFSRGNYRVSWPKFAVPNLQSLTNLLSSNLSWLSLDVSAAFYHLPLHPAAMPHLLVGSSGLSRYVARLSSNSRILNNQHGTMPDLHDYCSRNLYVSLLLLYQTFGRKLHLYSHPIILGFRKIPMGVGLSPFLLAQFTSAICSVVRRAFPHCLAFSYMDDVVLGAKSVQHLESLFTAVTNFLLSLGIHLNPNKTKRWGYSLNFMGYVIGCYGSLPQEHIIQKIKECFRKLPINRPIDWKVCQRIVGLLGFAAPFTQCGYPALMPLYACIQSKQAFTFSPTYKAFLCKQYLNLYPVARQRPGLCQVFADATPTGWGLVMGHQRMRGTFSAPLPIHTAELLAACFARSRSGANIIGTDNSVVLSRKYTSFPWLLGCAANWILRGTSFVYVPSALNPADDPSRGRLGLSRPLLRLPFRPTTGRTSLYADSPSVPSHLPDRVHFASPLHVAWRPP

SEQ ID NO: 33 - protein, 389 aa, Hepatitis B virus
  HBV S protein (YP_009173869)
MGQNLSTSNPLGFFPDHQLDPAFRANTANPDWDFNPNKDTWPDANKVGAGAFGLGFTPPHGGLLGWSPQAQGILQTLPANPPPASTNRQSGRQPTPLSPPLRNTHPQAMQWNSTTFHQTLQDPRVRGLYFPAGGSSSGTVNPVLTTASPLSSIFSRIGDPALNMENITSGFLGPLLVLQAGFFLLTRILTIPQSLDSWWTSLNFLGGTTVCLGQNSQSPTSNHSPTSCPPTCPGYRWMCLRRFIIFLFILLLCLIFLLVLLDYQGMLPVCPLIPGSSTTSTGPCRTCMTTAQGTSMYPSCCCTKPSDGNCTCIPIPSSWAFGKFLWEWASARFSWLSLLVPFVQWFVGLSPTVWLSVIWMMWYWGPSLYSILSPFLPLLPIFFCLWVYI

SEQ ID NO: 34 - protein, 281 aa, Hepatitis B virus
  HBV PreS2 protein (YP_009173870.1)
MQWNSTTFHQTLQDPRVRGLYFPAGGSSSGTVNPVLTTASPLSSIFSRIGDPALNMENITSGFLGPLLVLQAGFFLLTRILTIPQSLDSWWTSLNFLGGTTVCLGQNSQSPTSNHSPTSCPPTCPGYRWMCLRRFIIFLFILLLCLIFLLVLLDYQGMLPVCPLIPGSSTTSTGPCRTCMTTAQGTSMYPSCCCTKPSDGNCTCIPIPSSWAFGKFLWEWASARFSWLSLLVPFVQWFVGLSPTVWLSVIWMMWYWGPSLYSILSPFLPLLPIFFCLWVYI

SEQ ID NO: 35 - protein, 226 aa, Hepatitis B virus
  HBV S protein (YP_009173871.1)
MENITSGFLGPLLVLQAGFFLLTRILTIPQSLDSWWTSLNFLGGTTVCLGQNSQSPTSNHSPTSCPPTCPGYRWMCLRRFIIFLFILLLCLIFLLVLLDYQGMLPVCPLIPGSSTTSTGPCRTCMTTAQGTSMYPSCCCTKPSDGNCTCIPIPSSWAFGKFLWEWASARFSWLSLLVPFVQWFVGLSPTVWLSVIWMMWYWGPSLYSILSPFLPLLPIFFCLWVYI

SEQ ID NO: 36 - protein, 154 aa, Hepatitis B virus
  HBV X protein (YP_009173867.1)
MAARLCCQLDPARDVLCLRPVGAESCGRPFSGSLGTLSSPSPSAVPTDHGAHLSLRGLPVCAFSSAGPCALRFTSARRMETTVNAHQILPKVLHKRTLGLSAMSTTDLEAYFKDCLFKDWEELGEEIRLKVFVLGGCRHKLVCAPAPCNFFTSA

SEQ ID NO: 37 - protein, 212 aa, Hepatitis B virus
  HBV PreC protein (YP_009173857.1)
MQLFHLCLIISCSCPTVQASKLCLGWLWGMDIDPYKEFGATVELLSFLPSDFFPSVRDLLDTASALYREALESPEHCSPHHTALRQAILCWGELMTLATWVGVNLEDPASRDLVVSYVNTNMGLKFRQLLWFHISCLTFGRETVIEYLVSFGVWIRTPPAYRPPNAPILSTLPETTVVRRRGRSPRRRTPSPRRRRSQSPRRRRSQSRESQC

SEQ ID NO: 38 - protein, 843 aa, Hepatitis B virus
  HBV pol protein (BAA32913.1)
MPLSYQHFRKLLLLDDEAGPLEEELPRLADEGLNRRVAEDLNLGNLNVSIPWTHKVGNFTGLYSSTVPVFNPEWQTPSFPHIHLQEDIINRCQQYVGPLTVNEKRRLKLIMPARFYPNLTKYLPLDKGIKPYYPEHAVNHYFKTRHYLHTLWKAGILYKRETTRSASFCGSPYSWEQELQHGRLVFQTSTRHGDKSFCSQSSGILSRSPVGPCVRSQLKQSRLGLQPQQGSLARGKSGRSGSIRARVHPTTRRSFGVEPSGSGHIDNSASSTSSCLHQSAVRKTAYSHLSTSKRQSSSGHAVELHHIPPSSATPQSKGPILSCWWLQFRNSKPCSDYCLSHIVNLLEDWGPCTEHGEHNIRIPRTPARVTGGVFLVDKNPHNTTESRLVVDFSQFSRGSTHVSWPKFAVPNLQSLTNLLSSNLSWLSLDVSAAFYHIPLHPAAMPHLLVGSSGLPRYVARLSSTSRNINYQHGTMQDLHDSCSRHLYVSLLLLYKTFGRKLHLYSHPIILGFRKIPMGVGLSPFLLAQFTSAICSVVRRAFPHCLAFSYMDDVVLGAKSVQHLESLFTAVTNFLLSLGIHLNPNKTKRWGYSLNFMGYVIGSWGTLPQDHIVLKIKQCFRKLPVNRPIDWKVCQRIVGLLGFAAPFTQCGYPALMPLYACIQSKQAFTFSPTYKAFLCKQYLNLYPVARQRSGLCQVFADATPTGWGLAIGHRRMRGTFVAPLPIHTAELLAACFARSRSGAKLIGTDNSVVLSRKYTSFPWLLGCAANWILRGTSFVYVPSALNPADDPSRGRLGLYRPLLHLPFRPTTGRTSLYAVSPSVPSHLPDRVHFASPLHVAWRPP

SEQ ID NO: 39 - protein, 400 aa, Hepatitis B virus
  HBV envelope protein (BAA32914.1)
MGGWSSKPRQGMGTNLSVPNPLGFFPDHQLDPAFGANSNNPDWDFNPNKDHWPEANQVGAGAFGPGFTPPHGGLLGWSPQAQGTLTTVPVAPPPASTNRQSGRQPTPISPPLRDSHPQAMQWNSTTFHQALLHPRVRGLYFPAGGSSSGTVNPVPTTASPISSIFSRTGDPAPNMENTTSGFLGPLLVLQAGFFLLTRILTIPQSLDSWWTSLNFLGGAPTCPGQNSQSPTSNHSPTSCPPICPGYRWMCLRRFIIFLFILLLCLIFLLVLLDYQGMLPVCPLLPGTSTTSTGPCKTCTIPAQGTSMFPSCCCTKPSDGNCTCIPIPSSWAFARFLWEWASVRFSWLSLLVPFVQWFVGLSPTVWLSVIWMMWYWGPSLYNILSPFLPLLPIFFCLWVYI

SEQ ID NO: 40 - protein, 210 aa, Hepatitis B virus
  HBV X protein (BAA32912.1)
MGLGYWPSPHAWNLCGSSADPYCGTPSSLFCSQPVWSETDRNGQLCCSLSEIHLLSMAARVCCQLDPARDVLCLRPVGAESRGRPISGPFGSLPSPSSSAVPADHGAHLSLRGLPVCAFSSAGPCALRFTSARRMETTVNAHQVLPKVLYKRTLGLSAMSTTDLEAYFKDCLFKDWEELGEEIRLMIFVLGGCRHKLVCSPAPCNFFTSA

SEQ ID NO: 41 - protein, 389 aa, Hepatitis B virus; identical to SEQ ID NO: 33
  HBV Large S protein (P03138.3)

SEQ ID NO: 42 - protein, 183 aa, Hepatitis B virus
  HBV Core protein (P03146.1)
MDIDPYKEFGATVELLSFLPSDFFPSVRDLLDTASALYREALESPEHCSPHHTALRQAILCWGELMTLATWVGVNLEDPASRDLVVSYVNTNMGLKFRQLLWFHISCLTFGRETVIEYLVSFGVWIRTPPAYRPPNAPILSTLPETTVVRRRGRSPRRRTPSPRRRRSQSPRRRRSQSRESQC

SEQ ID NO: 43 - DNA, 3182 bp, Hepatitis B virus
  Hepatitis B virus (strain ayw) genome
aattccactgcatggcctgaggatgagtgtttctcaaaggtggagacagcggggtaggctgccttcctgactggcgattggtggaggcaggaggcggatttgctggcaaagtttgtagtatgccctgagcctgagggctccaccccaaaaggcctccgtgcggtggggtgaaacccagcccgaatgctccagctcctaccttgttggcgtctggccaggtgtccttgttgggattgaagtcccaatctggatttgcggtgtttgctctgaaggctggatccaactggtggtcgggaaagaatcccagaggattgctggtggaaagattctgccccatgctgtagatcttgttcccaagaatatggtgacccacaaaatgaggcgctatgtgttgtttctctcttatataatatacccgccttccatagagtgtgtaaatagtgtctagtttggaagtaatgattaactagatgttctggataataaggtttaatacccttatccaatggtaaatatttggtaacctttggataaaacctggcaggcataatcaattgcaatcttcttttctcattaactgtgagtgggcctacaaactgttcacattttttgataatgtcttggtgtaaatgtatattaggaaaagatggtgttttccaatgaggattaaagacaggtacagtagaagaataaagcccagtaaagttccccaccttatgagtccaaggaatactaacattgagattcccgagattgagatcttctgcgacgcggcgattgagaccttcgtctgcgaggcgagggagttcttcttctaggggacctgcctcgtcgtctaacaacagtagtctccggaagtgttgataggataggggcatttggtggtctataagctggaggagtgcgaatccacactccgaaagacaccaaatactctataactgtttctcttccaaaagtgagacaagaaatgtgaaaccacaagagttgcctgaactttaggcccatattagtgttgacataactgactactaggtctctagacgctggatcttccaaattaacacccacccaggtagctagagtcattagttccccccagcaaagaattgcttgcctgagtgcagtatggtgaggtgaacaatgctcaggagactctaaggcttcccgatacagagctgaggcggtatctagaagatctcgtactgaaggaaagaagtcagaaggcaaaaacgagagtaactccacagtagctccaaattctttataagggtcgatgtccatgccccaaagccacccaaggcacagcttggaggcttgaacagtaggacatgaacaagagatgattaggcagaggtgaaaaagttgcatggtgctggtgcgcagaccaatttatgcctacagcctcctagtacaaagacctttaacctaatctcctcccccaactcctcccagtctttaaacaaacagtctttgaagtatgcctcaaggtcggtcgttgacattgctgagagtccaagagtcctcttatgtaagaccttgggcaatatttggtgggcgttcacggtggtctccatgcgacgtgcagaggtgaagcgaagtgcacacggtccggcagatgagaaggcacagacggggagtccgcgtaaagagaggtgcgccccgtggtcggtcggaacggcagacggagaaggggacgagagagtcccaagcgaccccgagaagggtcgtccgcaggattcagcgccgacgggacgtaaacaaaggacgtcccgcgcaggatccagttggcagcacagcctagcagccatggaaacgatgtatatttgcgggataggacaacagagttatcagtcccgataatgtttgctccagacctgctgcgagcaaaacaagcggctaggagttccgcagtatggatcggcagaggagccgaaaaggttccacgcatgcgctgatggcccatgaccaagccccagccagtgggggttgcgtcagcaaacacttggcacagacctggccgttgccgggcaacggggtaaaggttcaggtattgtttacacagaaaggccttgtaagttggcgagaaagtgaaagcctgcttagattgaatacatgcatacaaaggcatcaacgcaggataaccacattgtgtaaaaggggcagcaaaacccaaaagacccacaattcgttgacatactttccaatcaataggcctgttaataggaagttttctaaaacattctttgattttttgtatgatgtgttcttgtggcaaggacccataacatccaatgacataacccataaaatttagagagtaaccccatctctttgttttgttagggtttaaatgtatacccaaagacaaaagaaaattggtaacagcggtaaaaagggactcaagatgctgtacagacttggcccccaataccacatcatccatataactgaaagccaaacagtgggggaaagccctacgaaccactgaacaaatggcactagtaaactgagccaggagaaacgggctgaggcccactcccataggaattttccgaaagcccaggatgatgggatgggaatacaggtgcaatttccgtccgaaggtttggtacagcaacaggagggatacatagaggttccttgagcagtagtcatgcaggtccggcatggtcccgtgctggttgttgaggatcctggaattagaggacaaacgggcaacataccttgatagtccagaagaaccaacaagaagatgaggcatagcagcaggatgaagaggaagatgataaaacgccgcagacacatccagcgataaccaggacaagttggaggacaagaggttggtgagtgattggaggttggggactgcgaattttggccaagacacacggtagttccccctagaaaattgagagaagtccaccacgagtctagactctgcggtattgtgaggattcttgtcaacaagaaaaaccccgcctgtaacacgagaaggggtcctaggaatcctgatgtgatgttctccatgttcagcgcagggtccccaatcctcgagaagattgacgataagggagaggcagtagtcagaacagggtttactgttcctgaactggagccaccagcagggaaatacaggcctctcactctgggatcttgcagagtttggtggaaggttgtgg

SEQ ID NO: 44 - DNA, 3182 bp, Artificial Sequence
  Reverse complement of SEQ ID NO: 16
ccacaaccttccaccaaactctgcaagatcccagagtgagaggcctgtatttccctgctggtggctccagttcaggaacagtaaaccctgttctgactactgcctctcccttatcgtcaatcttctcgaggattggggaccctgcgctgaacatggagaacatcacatcaggattcctaggaccccttctcgtgttacaggcggggtttttcttgttgacaagaatcctcacaataccgcagagtctagactcgtggtggacttctctcaattttctagggggaactaccgtgtgtcttggccaaaattcgcagtccccaacctccaatcactcaccaacctcttgtcctccaacttgtcctggttatcgctggatgtgtctgcggcgttttatcatcttcctcttcatcctgctgctatgcctcatcttcttgttggttcttctggactatcaaggtatgttgcccgtttgtcctctaattccaggatcctcaacaaccagcacgggaccatgccggacctgcatgactactgctcaaggaacctctatgtatccctcctgttgctgtaccaaaccttcggacggaaattgcacctgtattcccatcccatcatcctgggctttcggaaaattcctatgggagtgggcctcagcccgtttctcctggctcagtttactagtgccatttgttcagtggttcgtagggctttcccccactgtttggctttcagttatatggatgatgtggtattgggggccaagtctgtacagcatcttgagtccctttttaccgctgttaccaattttcttttgtctttgggtatacatttaaaccctaacaaaacaaagagatggggttactctctaaattttatgggttatgtcattggatgttatgggtccttgccacaagaacacatcatacaaaaaatcaaagaatgttttagaaaacttcctattaacaggcctattgattggaaagtatgtcaacgaattgtgggtcttttgggttttgctgccccttttacacaatgtggttatcctgcgttgatgcctttgtatgcatgtattcaatctaagcaggctttcactttctcgccaacttacaaggcctttctgtgtaaacaatacctgaacctttaccccgttgcccggcaacggccaggtctgtgccaagtgtttgctgacgcaacccccactggctggggcttggtcatgggccatcagcgcatgcgtggaaccttttcggctcctctgccgatccatactgcggaactcctagccgcttgttttgctcgcagcaggtctggagcaaacattatcgggactgataactctgttgtcctatcccgcaaatatacatcgtttccatggctgctaggctgtgctgccaactggatcctgcgcgggacgtcctttgtttacgtcccgtcggcgctgaatcctgcggacgacccttctcggggtcgcttgggactctctcgtccccttctccgtctgccgttccgaccgaccacggggcgcacctctctttacgcggactccccgtctgtgccttctcatctgccggaccgtgtgcacttcgcttcacctctgcacgtcgcatggagaccaccgtgaacgcccaccaaatattgcccaaggtcttacataagaggactcttggactctcagcaatgtcaacgaccgaccttgaggcatacttcaaagactgtttgtttaaagactgggaggagttgggggaggagattaggttaaaggtctttgtactaggaggctgtaggcataaattggtctgcgcaccagcaccatgcaactttttcacctctgcctaatcatctcttgttcatgtcctactgttcaagcctccaagctgtgccttgggtggctttggggcatggacatcgacccttataaagaatttggagctactgtggagttactctcgtttttgccttctgacttctttccttcagtacgagatcttctagataccgcctcagctctgtatcgggaagccttagagtctcctgagcattgttcacctcaccatactgcactcaggcaagcaattctttgctggggggaactaatgactctagctacctgggtgggtgttaatttggaagatccagcgtctagagacctagtagtcagttatgtcaacactaatatgggcctaaagttcaggcaactcttgtggtttcacatttcttgtctcacttttggaagagaaacagttatagagtatttggtgtctttcggagtgtggattcgcactcctccagcttatagaccaccaaatgcccctatcctatcaacacttccggagactactgttgttagacgacgaggcaggtcccctagaagaagaactccctcgcctcgcagacgaaggtctcaatcgccgcgtcgcagaagatctcaatctcgggaatctcaatgttagtattccttggactcataaggtggggaactttactgggctttattcttctactgtacctgtctttaatcctcattggaaaacaccatcttttcctaatatacatttacaccaagacattatcaaaaaatgtgaacagtttgtaggcccactcacagttaatgagaaaagaagattgcaattgattatgcctgccaggttttatccaaaggttaccaaatatttaccattggataagggtattaaaccttattatccagaacatctagttaatcattacttccaaactagacactatttacacactctatggaaggcgggtatattatataagagagaaacaacacatagcgcctcattttgtgggtcaccatattcttgggaacaagatctacagcatggggcagaatctttccaccagcaatcctctgggattctttcccgaccaccagttggatccagccttcagagcaaacaccgcaaatccagattgggacttcaatcccaacaaggacacctggccagacgccaacaaggtaggagctggagcattcgggctgggtttcaccccaccgcacggaggccttttggggtggagccctcaggctcagggcatactacaaactttgccagcaaatccgcctcctgcctccaccaatcgccagtcaggaaggcagcctaccccgctgtctccacctttgagaaacactcatcctcaggccatgcagtggaatt

SEQ ID NO: 45 - protein, 389 aa, Hepatitis B virus
  HBV S protein (P03142.4)
MGTNLSVPNPLGFLPDHQLDPAFGANSTNPDWDFNPIKDHWPAANQVGVGAFGPGLTPPHGGILGWSPQAQGILTTVSTIPPPASTNRQSGRQPTPISPPLRDSHPQAMQWNSTALHQALQDPRVRGLYLPAGGSSSGTVNPAPNIASHISSISARTGDPVTIMENITSGFLGPLLVLQAGFFLLTRILTIPQSLDSWWTSLNFLGGSPVCLGQNSQSPTSNHSPTSCPPICPGYRWMCLRRFIIFLFILLLCLIFLLVLLDYQGMLPVCPLIPGSTTTSTGPCKTCTTPAQGNSKFPSCCCTKPTDGNCTCIPIPSSWAFAKYLWEWASVRFSWLSLLVPFVQWFVGLSPTVWLSAIWMMWYWGPSLYSIVSPFIPLLPIFFCLWVYI

SEQ ID NO: 46 - protein, 185 aa, Hepatitis B virus
  HBV Core protein (P03149.1)
MDIDPYKEFGATVELLSFLPSDFFPSVRDLLDTASALYREALESPEHCSPHHTALRQAILCWGELMTLATWVGNNLQDPASRDLVVNYVNTNMGLKIRQLLWFHISCLTFGRETVLEYLVSFGVWIRTPPAYRPPNAPILSTLPETTVVRRRDRGRSPRRRTPSPRRRRSQSPRRRRSQSRESQC

SEQ ID NO: 47 - DNA, 3200 bp, Hepatitis B virus
  Hepatitis B virus complete DNA sequence (subtype adw)
ttccactgccttgcaccaagctctgcaggatcccagagtcaggggtctgtatcttcctgctggtggctccagttcaggaacagtaaaccctgctccgaatattgcctctcacatctcgtcaatctccgcgaggactggggaccctgtgacgatcatggagaacatcacatcaggattcctaggacccctgctcgtgttacaggcggggtttttcttgttgacaagaatcctcacaataccgcagagtctagactcgtggtggacttctctcaattttctagggggatcacccgtgtgtcttggccaaaattcgcagtccccaacctccaatcactcaccaacctcctgtcctccaatttgtcctggttatcgctggatgtgtctgcggcgttttatcatattcctcttcatcctgctgctatgcctcatcttcttattggttcttctggattatcaaggtatgttgcccgtttgtcctctaattccaggatcaacaacaaccagtacgggaccatgcaaaacctgcacgactcctgctcaaggcaactctaagtttccctcatgttgctgtacaaaacctacggatggaaattgcacctgtattcccatcccatcgtcctgggctttcgcaaaatacctatgggagtgggcctcagtccgtttctcttggctcagtttactagtgccatttgttcagtggttcgtagggctttcccccactgtttggctttcagctatatggatgatgtggtattgggggccaagtctgtacagcatcgtgagtccctttataccgctgttaccaattttcttttgtctctgggtatacatttaaaccctaacaaaacaaaaagatggggttattccctaaacttcatgggctacataattggaagttggggaactttgccacaggatcatattgtacaaaagatcaaacactgttttagaaaacttcctgttaacaggcctattgattggaaagtatgtcaaagaattgtgggtcttttgggctttgctgctccatttacacaatgtggatatcctgccttaatgcctttgtatgcatgtatacaagctaaacaggctttcactttctcgccaacttacaaggcctttctaagtaaacagtacatgaacctttaccccgttgctcggcaacggcctggtctgtgccaagtgtttgctgacgcaacccccactggctggggcttagccataggccatcagcgcatgcgtggaacctttgtggctcctctgccgatccatactgcggaactcctagccgcttgttttgctcgcagccggtctggagcaaagctcatcggaactgacaattctgtcgtcctctcgcggaaatatacatcatttccatggctgctaggctgtactgccaactggatccttcgcgggacgtcctttgtttacgtcccgtcggcgctgaatcccgcggacgacccctctcggggccgcttgggactctctcgtccccttctccgtctgccgttccagccgaccacggggcgcacctctctttacgcggtctccccgtctgtgccttctcatctgccggtccgtgtgcacttcgcttcacctctgcacgttgcatggcgaccaccgtgaacgcccatcagatcctgcccaaggtcttacataagaggactcttggactcccagcaatgtcaacgaccgaccttgaggcctacttcaaagactgtgtgtttaaggactgggaggagttgggggaggagattaggttaatgatctttgtattaggaggctgtaggcataaattggtctgcgcaccagcaccatgcaactttttcacctctgcctaatcatctcttgtacatgtcccactgttcaagcctccaagctgtgccttgggtggctttggggcatggacattgacccttataaagaatttggagctactgtggagttactctcgtttttgccttctgacttctttccttccgtacgagatctcctagacaccgcctcagctctgtatcgagaagccttagagtctcctgagcattgctcacctcaccatactgcactcaggcaagccattctctgctggggggaattgatgactctagctacctgggtgggtaataatttgcaagatccagcatccagagatctagtagtcaattatgttaatactaacatgggtttaaagatcaggcaactattgtggtttcatatatcttgccttacttttggaagagagactgtacttgaatatttggtctctttcggagtgtggattcgcactcctccagcctatagaccaccaaatgcccctatcttatcaacacttccggaaactactgttgttagacgacgggaccgaggcaggtcccctagaagaagaactccctcgcctcgcagacgcagatctcaatcgccgcgtcgcagaagatctcaatctcgggaatctcaatgttagtattccttggactcataaggtcggaaactttacggggctttattcctctacagtacctatctttaatcctgaatggcaaactccttcctttcctaagattcatttacaagaggacattattaataggtgtcaacaatttgtgggccctctcactgtaaatgaaaagagaagattgaaattaattatgcctgctagattctatcctacccacactaaatatttgcccttagacaaaggaattaaaccttattatccagatcaggtagttaatcattacttccaaaccagacattatttacatactctttggaaggctggtattctatataagagggaaaccacacgtagcgcatcattttgcgggtcaccatattcttgggaacaagagctacagcattcgcaaaggcatggggacgaatctttctgttcccaaccctctgggattccttcccgatcatcagttggaccctgcattcggagccaactcaacaaatccagattgggacttcaaccccatcaaggaccactggccagcagccaaccaggtaggagtgggagcattcgggccagggctcacccctccacacggcggtattttggggtggagccctcaggctcagggcatattgaccacagtgtcaacaattcctcctcctgcctccaccaatcggcagtcaggaaggcagcctactcccatctctccacctctaagagacagtcatcctcaggccatgcagtggaa

SEQ ID NO: 48 - DNA, 3200 bp, Artificial Sequence
  Reverse complement of SEQ ID NO: 47
ttccactgcatggcctgaggatgactgtctcttagaggtggagagatgggagtaggctgccttcctgactgccgattggtggaggcaggaggaggaattgttgacactgtggtcaatatgccctgagcctgagggctccaccccaaaataccgccgtgtggaggggtgagccctggcccgaatgctcccactcctacctggttggctgctggccagtggtccttgatggggttgaagtcccaatctggatttgttgagttggctccgaatgcagggtccaactgatgatcgggaaggaatcccagagggttgggaacagaaagattcgtccccatgcctttgcgaatgctgtagctcttgttcccaagaatatggtgacccgcaaaatgatgcgctacgtgtggtttccctcttatatagaataccagccttccaaagagtatgtaaataatgtctggtttggaagtaatgattaactacctgatctggataataaggtttaattcctttgtctaagggcaaatatttagtgtgggtaggatagaatctagcaggcataattaatttcaatcttctcttttcatttacagtgagagggcccacaaattgttgacacctattaataatgtcctcttgtaaatgaatcttaggaaaggaaggagtttgccattcaggattaaagataggtactgtagaggaataaagccccgtaaagtttccgaccttatgagtccaaggaatactaacattgagattcccgagattgagatcttctgcgacgcggcgattgagatctgcgtctgcgaggcgagggagttcttcttctaggggacctgcctcggtcccgtcgtctaacaacagtagtttccggaagtgttgataagataggggcatttggtggtctataggctggaggagtgcgaatccacactccgaaagagaccaaatattcaagtacagtctctcttccaaaagtaaggcaagatatatgaaaccacaatagttgcctgatctttaaacccatgttagtattaacataattgactactagatctctggatgctggatcttgcaaattattacccacccaggtagctagagtcatcaattccccccagcagagaatggcttgcctgagtgcagtatggtgaggtgagcaatgctcaggagactctaaggcttctcgatacagagctgaggcggtgtctaggagatctcgtacggaaggaaagaagtcagaaggcaaaaacgagagtaactccacagtagctccaaattctttataagggtcaatgtccatgccccaaagccacccaaggcacagcttggaggcttgaacagtgggacatgtacaagagatgattaggcagaggtgaaaaagttgcatggtgctggtgcgcagaccaatttatgcctacagcctcctaatacaaagatcattaacctaatctcctcccccaactcctcccagtccttaaacacacagtctttgaagtaggcctcaaggtcggtcgttgacattgctgggagtccaagagtcctcttatgtaagaccttgggcaggatctgatgggcgttcacggtggtcgccatgcaacgtgcagaggtgaagcgaagtgcacacggaccggcagatgagaaggcacagacggggagaccgcgtaaagagaggtgcgccccgtggtcggctggaacggcagacggagaaggggacgagagagtcccaagcggccccgagaggggtcgtccgcgggattcagcgccgacgggacgtaaacaaaggacgtcccgcgaaggatccagttggcagtacagcctagcagccatggaaatgatgtatatttccgcgagaggacgacagaattgtcagttccgatgagctttgctccagaccggctgcgagcaaaacaagcggctaggagttccgcagtatggatcggcagaggagccacaaaggttccacgcatgcgctgatggcctatggctaagccccagccagtgggggttgcgtcagcaaacacttggcacagaccaggccgttgccgagcaacggggtaaaggttcatgtactgtttacttagaaaggccttgtaagttggcgagaaagtgaaagcctgtttagcttgtatacatgcatacaaaggcattaaggcaggatatccacattgtgtaaatggagcagcaaagcccaaaagacccacaattctttgacatactttccaatcaataggcctgttaacaggaagttttctaaaacagtgtttgatcttttgtacaatatgatcctgtggcaaagttccccaacttccaattatgtagcccatgaagtttagggaataaccccatctttttgttttgttagggtttaaatgtatacccagagacaaaagaaaattggtaacagcggtataaagggactcacgatgctgtacagacttggcccccaataccacatcatccatatagctgaaagccaaacagtgggggaaagccctacgaaccactgaacaaatggcactagtaaactgagccaagagaaacggactgaggcccactcccataggtattttgcgaaagcccaggacgatgggatgggaatacaggtgcaatttccatccgtaggttttgtacagcaacatgagggaaacttagagttgccttgagcaggagtcgtgcaggttttgcatggtcccgtactggttgttgttgatcctggaattagaggacaaacgggcaacataccttgataatccagaagaaccaataagaagatgaggcatagcagcaggatgaagaggaatatgataaaacgccgcagacacatccagcgataaccaggacaaattggaggacaggaggttggtgagtgattggaggttggggactgcgaattttggccaagacacacgggtgatccccctagaaaattgagagaagtccaccacgagtctagactctgcggtattgtgaggattcttgtcaacaagaaaaaccccgcctgtaacacgagcaggggtcctaggaatcctgatgtgatgttctccatgatcgtcacagggtccccagtcctcgcggagattgacgagatgtgagaggcaatattcggagcagggtttactgttcctgaactggagccaccagcaggaagatacagacccctgactctgggatcctgcagagcttggtgcaaggcagtggaa

SEQ ID NO: 49 - DNA, 3182 bp, Hepatitis B virus
  Hepatitis B virus subtype ayw, complete genome
aattccacaacctttcaccaaactctgcaagatcccagagtgagaggcctgtatttccctgctggtggctccagttcaggagcagtaaaccctgttccgactactgcctctcccttatcgtcaatcttctcgaggattggggaccctgcgctgaacatggagaacatcacatcaggattcctaggaccccttctcgtgttacaggcggggtttttcttgttgacaagaatcctcacaataccgcagagtctagactcgtggtggacttctctcaattttctagggggaactaccgtgtgtcttggccaaaattcgcagtccccaacctccaatcactcaccaacctcctgtcctccaacttgtcctggttatcgctggatgtgtctgcggcgttttatcatcttcctcttcatcctgctgctatgcctcatcttcttgttggttcttctggactatcaaggtatgttgcccgtttgtcctctaattccaggatcctcaaccaccagcacgggaccatgccgaacctgcatgactactgctcaaggaacctctatgtatccctcctgttgctgtaccaaaccttcggacggaaattgcacctgtattcccatcccatcatcctgggctttcggaaaattcctatgggagtgggcctcagcccgtttctcctggctcagtttactagtgccatttgttcagtggttcgtagggctttcccccactgtttggctttcagttatatggatgatgtggtattgggggccaagtctgtacagcatcttgagtccctttttaccgctgttaccaattttcttttgtctttgggtatacatttaaaccctaacaaaacaaagagatggggttactctctgaattttatgggttatgtcattggaagttatgggtccttgccacaagaacacatcatacaaaaaatcaaagaatgttttagaaaacttcctattaacaggcctattgattggaaagtatgtcaacgaattgtgggtcttttgggttttgctgccccatttacacaatgtggttatcctgcgttaatgcccttgtatgcatgtattcaatctaagcaggctttcactttctcgccaacttacaaggcctttctgtgtaaacaatacctgaacctttaccccgttgcccggcaacggccaggtctgtgccaagtgtttgctgacgcaacccccactggctggggcttggtcatgggccatcagcgcgtgcgtggaaccttttcggctcctctgccgatccatactgcggaactcctagccgcttgttttgctcgcagcaggtctggagcaaacattatcgggactgataactctgttgtcctctcccgcaaatatacatcgtatccatggctgctaggctgtgctgccaactggatcctgcgcgggacgtcctttgtttacgtcccgtcggcgctgaatcctgcggacgacccttctcggggtcgcttgggactctctcgtccccttctccgtctgccgttccgaccgaccacggggcgcacctctctttacgcggactccccgtctgtgccttctcatctgccggaccgtgtgcacttcgcttcacctctgcacgtcgcatggagaccaccgtgaacgcccaccgaatgttgcccaaggtcttacataagaggactcttggactctctgcaatgtcaacgaccgaccttgaggcatacttcaaagactgtttgtttaaagactgggaggagttgggggaggagattagattaaaggtctttgtactaggaggctgtaggcataaattggtctgcgcaccagcaccatgcaactttttcacctctgcctaatcatctcttgttcatgtcctactgttcaagcctccaagctgtgccttgggtggctttggggcatggacatcgacccttataaagaatttggagctactgtggagttactctcgtttttgccttctgacttctttccttcagtacgagatcttctagataccgcctcagctctgtatcgggaagccttagagtctcctgagcattgttcacctcaccatactgcactcaggcaagcaattctttgctggggggaactaatgactctagctacctgggtgggtgttaatttggaagatccagcatctagagacctagtagtcagttatgtcaacactaatatgggcctaaagttcaggcaactcttgtggtttcacatttcttgtctcacttttggaagagaaaccgttatagagtatttggtgtctttcggagtgtggattcgcactcctccagcttatagaccaccaaatgcccctatcctatcaacacttccggaaactactgttgttagacgacgaggcaggtcccctagaagaagaactccctcgcctcgcagacgaaggtctcaatcgccgcgtcgcagaagatctcaatctcgggaacctcaatgttagtattccttggactcataaggtggggaactttactggtctttattcttctactgtacctgtctttaatcctcattggaaaacaccatcttttcctaatatacatttacaccaagacattatcaaaaaatgtgaacagtttgtaggcccacttacagttaatgagaaaagaagattgcaattgattatgcctgctaggttttatccaaaggttaccaaatatttaccattggataagggtattaaaccttattatccagaacatctagttaatcattacttccaaactagacactatttacacactctatggaaggcgggtatattatataagagagaaacaacacatagcgcctcattttgtgggtcaccatattcttgggaacaagatctacagcatggggcagaatctttccaccagcaatcctctgggattctttcccgaccaccagttggatccagccttcagagcaaacacagcaaatccagattgggacttcaatcccaacaaggacacctggccagacgccaacaaggtaggagctggagcattcgggctgggtttcaccccaccgcacggaggccttttggggtggagccctcaggctcagggcatactacaaactttgccagcaaatccgcctcctgcctccaccaatcgccagacaggaaggcagcctaccccgctgtctccacctttgagaaacactcatcctcaggccatgcagtgg